European Patent Application EP 4 186 564 A1, published May 31, 2023. Title: MULTISPECIFIC HEAVY CHAIN ANTIBODIES WITH MODIFIED HEAVY CHAIN CONSTANT REGIONS. Applicant: TeneoBio, Inc. Application EP EP22203885, filed April 29, 2021. The sequence listing filed with the application follows.

SEQUENCE LISTING (93 sequences)

SEQ ID NO: 1 - protein, 120 aa, synthetic construct
  REGION 1..120: note = source = /note="Description of Artificial Sequence: Syntheticpolypeptide"
QLQLQESGPGLVKPSETLSLTCTVSGGSISSSSYYWGWIRQPPGKGLEWIGSIDYSGYTYYNPSLQSRVTISVDTSKNQFSLKLSSVTAADTAVYNCARHKAATADFDYRGQGTLVTVSS

SEQ ID NO: 2 - protein, 120 aa, synthetic construct
  REGION 1..120: note = source = /note="Description of Artificial Sequence: Syntheticpolypeptide"
QLQLQESGPGLVKPSETLSLTCTVSGGSISSSNYFWGWIRQSPGKGLEWIGSIDYSGYTYYNPSLKSRVTISVDTSKNQFSLKLSSVTAADTAVYNCARHKAATADFDYRGQGTLVTVSS

SEQ ID NO: 3 - protein, 120 aa, synthetic construct
  REGION 1..120: note = source = /note="Description of Artificial Sequence: Syntheticpolypeptide"
QLQLQESGPGLVKPSETLSLTCTVSGGSISSSSYYWGWIRQPPGKGLEWIGSVDYSGYTYYNPSLQSRVTISVDTSKNQFSLKLSSVTAADTAVYNCARHKAATADFDYRGQGTLVTVSS

SEQ ID NO: 4 - protein, 120 aa, synthetic construct
  REGION 1..120: note = source = /note="Description of Artificial Sequence: Syntheticpolypeptide"
QLQLQESGPGLVKPSETLSLTCTVSGGSISSSSYYWGWIRQPPGKGLEWIGSIDYSGYTYYNPSLKSRVTISVDTSKNQFSLKLSSVTAADTAVYNCARHKAATADFDYRGQGTLVTVSS

SEQ ID NO: 5 - protein, 120 aa, synthetic construct
  REGION 1..120: note = source = /note="Description of Artificial Sequence: Syntheticpolypeptide"
QLQLQESGPGLVKPSETLSLTCTVSGGSISSNSYYWGWIRQSPGKGLEWLGSIYDSGSTHYNPSLKSRVIISGDTSKNQFSLKLSSVTAADTAVYYCARHKAATADFDYRGQGTLVTVSS

SEQ ID NO: 6 - protein, 127 aa, synthetic construct
  REGION 1..127: note = source = /note="Description of Artificial Sequence: Syntheticpolypeptide"
QVQLVESGGGVVQPGRSLRLSCAASGFSFRSYGMHWVRQAPGKGLEWVAVIWYDGSNKYYADSVKGRFTISRDYSKNTLYLQMNSLRAEDTAVYYCAREPRIGYYYESSGYDSLDYRGQGTLVTVSS

SEQ ID NO: 7 - protein, 127 aa, synthetic construct
  REGION 1..127: note = source = /note="Description of Artificial Sequence: Syntheticpolypeptide"
QVQLVESGGGVVQPGRSLRLSCAASGFSFSSYGMHWVRQAPGKGLEWVAVIWYDGSNKYYADSVKGRFTISRDYSKNTLYLQMNSLRAEDTAVYYCAREPRIGYYYESSGYDSLDYRGQGTLVTVSS

SEQ ID NO: 8 - protein, 127 aa, synthetic construct
  REGION 1..127: note = source = /note="Description of Artificial Sequence: Syntheticpolypeptide"
QVQLVESGGGVVQPGRSLRLSCAASGFSFSSYGMHWVRQAPGKGLEGVAVIWYDGSNRYYADSVKGRFTISRDNSKNTLYLQMNSLRAEDTAVYYCAREPRIGYYYESSGYYSLDYRGQGTLVTVSS

SEQ ID NO: 9 - protein, 127 aa, synthetic construct
  REGION 1..127: note = source = /note="Description of Artificial Sequence: Syntheticpolypeptide"
QVQLVESGGGVVQPGRSLRLSCAASGFIFRSYGMHWVRQAPGKGPEWVAVIWYDGSNKYYADSVKGRFTISRDNSKNTLYLQMNSLRAEDTAVYYCAREPRIGYYYESSGYYSLDYRGQGTLVTVSS

SEQ ID NO: 10 - protein, 127 aa, synthetic construct
  REGION 1..127: note = source = /note="Description of Artificial Sequence: Syntheticpolypeptide"
QVQLVESGGGVVQPGRSLRLSCAASGFSFRSYGMHWVRQAPGKGLEWVAVIWYDGSNKYYADSVKGRFTISRDYSKNTLYLQMNSLRAEDTAVYYCAREPRIGYYYDSSGYDSLDYRGQGTLVTVSS

SEQ ID NO: 11 - protein, 127 aa, synthetic construct
  REGION 1..127: note = source = /note="Description of Artificial Sequence: Syntheticpolypeptide"
QVQLVESGGGVVQPGRSLRLSCAASGFSFRSYGMHWVRQAPGKGLEWVAVIWYDGSNKYYADSVKGRFTISRDNSKNTLYLQMNSLRAEDTAVYYCAREPRIGYYYDSSGYDSLDYRGQGTLVTVSS

SEQ ID NO: 12 - protein, 127 aa, synthetic construct
  REGION 1..127: note = source = /note="Description of Artificial Sequence: Syntheticpolypeptide"
QVQLVESGGGVVQPGRSLRLSCAASGFIFRSYGMHWVRQAPGKGPEWVAVIWYDGSNKYYADSVKGRFTISRDNSKNTLYLQMNSLRAEDTAVYYCAREPRIGYYYDSSGYDSLDYRGQGTLVTVSS

SEQ ID NO: 13 - protein, 127 aa, synthetic construct
  REGION 1..127: note = source = /note="Description of Artificial Sequence: Syntheticpolypeptide"
QVQLVESGGGVVQPGRSLRLSCAASGFSFSSYGMHWVRQAPGKGLEGVAVIWYDGSNRYYADSVKGRFTISRDNSKNTLYLQMNSLRAEDTAVYYCAREPRIGYYYDSSGYYSLDYRGQGTLVTVSS

SEQ ID NO: 14 - protein, 127 aa, synthetic construct
  REGION 1..127: note = source = /note="Description of Artificial Sequence: Syntheticpolypeptide"
QVQLVESGGGVVQPGRSLRLSCAASGFSFRSYGMHWVRQAPGKGLEWVAVISYDGSNKYYADSVKGRFTISRDYSKNTLYLQMNSLRAEDTAVYYCAREPRIGYYYDSSGYDSLDYRGQGTLVTVSS

SEQ ID NO: 15 - protein, 127 aa, synthetic construct
  REGION 1..127: note = source = /note="Description of Artificial Sequence: Syntheticpolypeptide"
QVQLVESGGGVVQPGRSLRLSCAASGFSFSRYGMHWVRQAPGKGLEGVAVIWYDGSNRYYADSVKGRFTISRDNSKNTLYLQMNSLRAEDTAVYYCAREPRIGYYYESSGYYSLDYRGQGTLVTVSS

SEQ ID NO: 16 - protein, 127 aa, synthetic construct
  REGION 1..127: note = source = /note="Description of Artificial Sequence: Syntheticpolypeptide"
QVQLVESGGGVVQPGRSLRLSCAASGFSFSRYGMHWVRQAPGKGLEWVAVISYDGSNKYYADSVKGRFTISRDNSKNTLYLQMNSLRAEDTAVYYCAREPRVGYYYETSGYYSLDYRGQGTLVTVSS

SEQ ID NO: 17 - protein, 127 aa, synthetic construct
  REGION 1..127: note = source = /note="Description of Artificial Sequence: Syntheticpolypeptide"
QVQLVESGGGVVQPGRSLRLSCAASGFSFTSYGMHWVRQAPGKGLEGVAVIWYDGSNRYYADSVKGRFTISRDNSKNTLYLQMNSLRAEDTAVYYCAREPRIGYYYESSGYYSLDYRGQGTLVTVSS

SEQ ID NO: 18 - protein, 127 aa, synthetic construct
  REGION 1..127: note = source = /note="Description of Artificial Sequence: Syntheticpolypeptide"
QVQLVESGGGVVQPGRSLRLSCAASGFSFSRYGMHWVRQAPGKGLEWVAVIWYDGSNRYYADSVKGRFTISRDNSKNTLYLQMNSLRAEDTAVYYCAREPRIGYYYESSGYYSLDYRGQGTLVTVSS

SEQ ID NO: 19 - protein, 127 aa, synthetic construct
  REGION 1..127: note = source = /note="Description of Artificial Sequence: Syntheticpolypeptide"
QVQLVESGGGVVQPGRSLRLSCAASGFSFSRYGMHWVRQAPGKGLEGVAVIWYDGSNKYYADSVKGRFTISRDNSKNTLYLQMNSLRAEDTAVYYCAREPRIGYYYESSGYYSLDYRGQGTLVTVSS

SEQ ID NO: 20 - protein, 127 aa, synthetic construct
  REGION 1..127: note = source = /note="Description of Artificial Sequence: Syntheticpolypeptide"
QVQLVESGGGVVQPGRSLRLSCAASGFSFSSYGMHWVRQAPGKGLEGVAVIWYDGSNRYYADSVKGRFTISRDNSKNTLFLQMNSLRAEDTAVYYCAREPRIGYYYESSGYYSLDYRGQGTLVTVSS

SEQ ID NO: 21 - protein, 127 aa, synthetic construct
  REGION 1..127: note = source = /note="Description of Artificial Sequence: Syntheticpolypeptide"
QVQLVESGGGLVKPGGSLRLSCAASGFSFSSYGMHWVRQAPGKGLEGVAVIWYDGSNRYYADSVKGRFTISRDNSKNTLYLQMNSLRAEDTAVYYCAREPRIGYYYESSGYYSLDYRGQGTLVTVSS

SEQ ID NO: 22 - protein, 127 aa, synthetic construct
  REGION 1..127: note = source = /note="Description of Artificial Sequence: Syntheticpolypeptide"
QVQLVESGGGVVQPGRSLRLSCAASGFSFSSYGMHWVRQAPGKGLEGVAVIWYDGSNRYYADSVKGRFTISRDSSKNTLYLQMNSLRAEDTAVYYCAREPRIGYYYESSGYYSLDYRGQGTLVTVSS

SEQ ID NO: 23 - protein, 127 aa, synthetic construct
  REGION 1..127: note = source = /note="Description of Artificial Sequence: Syntheticpolypeptide"
QVQLVESGGGVVQPGRSLRLSCAASGFSFRSYGMHWVRQAPGKGLEWVAVIWYDGSNKYYADSVKGRFTISRDNSKNTMYLQMNSLRAEDTAVYYCAREPRIGYYYESSGYYSLDYRGQGTLVTVSS

SEQ ID NO: 24 - protein, 127 aa, synthetic construct; identical to SEQ ID NO: 9
  REGION 1..127: note = source = /note="Description of Artificial Sequence: Syntheticpolypeptide"

SEQ ID NO: 25 - protein, 127 aa, synthetic construct; identical to SEQ ID NO: 8
  REGION 1..127: note = source = /note="Description of Artificial Sequence: Syntheticpolypeptide"

SEQ ID NO: 26 - protein, 127 aa, synthetic construct
  REGION 1..127: note = source = /note="Description of Artificial Sequence: Syntheticpolypeptide"
QVQLVESGGGVVQPGRSLRLSCAASGFTFISYGMHWVRQAPGKGLEGVAVIWYDGSNRYYADSVKGRFTISRDNSKNTLYLQMNSLRAEDTAVYYCAREPRIGYYYESSGYYSLDYRGQGTLVTVSS

SEQ ID NO: 27 - protein, 127 aa, synthetic construct
  REGION 1..127: note = source = /note="Description of Artificial Sequence: Syntheticpolypeptide"
QVQLVESGGGVVQPGRSLRLSCAASGFSFSSYGMHWVRQAPGKGPEWVAVIWYDGSNRYYADSVKGRFTISRDNSKNTLYLQMNSLRAEDTAVYYCAREPRIGYYYESSGYYSLDYRGQGTLVTVSS

SEQ ID NO: 28 - protein, 127 aa, synthetic construct
  REGION 1..127: note = source = /note="Description of Artificial Sequence: Syntheticpolypeptide"
QVQLVESGGGVVQPGRSLRLSCAASGFSFSSYGMHWVRQAPGKGLEWVAVIWYDGSNRYYADSVKGRFTISRDNSKNTLYLQMNSLRAEDTAVYYCAREPRIGYYYESSGYYSLDYRGQGTLVTVSS

SEQ ID NO: 29 - protein, 127 aa, synthetic construct
  REGION 1..127: note = source = /note="Description of Artificial Sequence: Syntheticpolypeptide"
QVQLVESGGGVVQPGRSLRLSCAASGFSFSRYGMHWVRQAPGKGLEGVAVISYDGSNKYYADSVKGRFTISRDYSKNTLYLQMNSLRAEDTAVYYCAREPRIGYYYDSSGYDSLDYRGQGTLVTVSS

SEQ ID NO: 30 - protein, 127 aa, synthetic construct
  REGION 1..127: note = source = /note="Description of Artificial Sequence: Syntheticpolypeptide"
QVQLVESGGGLVQPGGSLRLSCAASGFSFSSYGMHWVRQAPGKGLEGVAVIWYDGSNKYYADSVKGRFTISRDNSKNTMYLQMNSLRAEDTAVYYCAREPRIGYYYESSGYYSLDYRGQGTLVTVSS

SEQ ID NO: 31 - protein, 127 aa, synthetic construct
  REGION 1..127: note = source = /note="Description of Artificial Sequence: Syntheticpolypeptide"
QVQLVESGGGVVQPGRSLRLSCAASGFTFSSYGMHWVRQAPGKGLEGVAVIWYDGSNRYYADSVKGRFTISRDNSKNTLYLQMNSLRAEDTAVYYCAREPRIGYYYESSGYYSLDYRGQGTLVTVSS

SEQ ID NO: 32 - protein, 127 aa, synthetic construct
  REGION 1..127: note = source = /note="Description of Artificial Sequence: Syntheticpolypeptide"
QVQLVESVGGVVQPGRSLRLSCAASGFSFSSYGMHWVRQAPGKGLEGVAVIWYDGSNRYYADSVKGRFTISRDNSKNTLYLQMNSLRAEDTAVYYCAREPRIGYYYESSGYYSLDYRGQGTLVTVSS

SEQ ID NO: 33 - protein, 127 aa, synthetic construct
  REGION 1..127: note = source = /note="Description of Artificial Sequence: Syntheticpolypeptide"
QVQLVESGGGVVQPGRSLRLSCAASGFSFSSYGMHWVRQAPGKGLEGVAVISYDGSNRYYADSVKGRFTISRDNSKNTLYLQMNSLRAEDTAVYYCAREPRIGYYYESSGYYSLDYRGQGTLVTVSS

SEQ ID NO: 34 - protein, 127 aa, synthetic construct
  REGION 1..127: note = source = /note="Description of Artificial Sequence: Syntheticpolypeptide"
QVQLVESGGGVVQPGRSLRLSCAASGFSFSSYGMHWVRQAPGKGLEWVAVIWYDGSNKYYADSVKGRFTISRDNSKNTMYLQMNSLRAEDTAVYYCAREPRIGYYYESSGYYSLDYRGQGTLVTVSS

SEQ ID NO: 35 - protein, 127 aa, synthetic construct
  REGION 1..127: note = source = /note="Description of Artificial Sequence: Syntheticpolypeptide"
QVQLVESGGGVVQPGRSLRLSCAASGFSFSSYGMHWVRQAPGKGPEWVAVIWYDGSNKYYADSVKGRFTISRDNSKNTLYLQMNSLRAEDTAVYYCAREPRIGYYYESSGYYSLDYRGQGTLVTVSS

SEQ ID NO: 36 - protein, 8 aa, synthetic construct
  REGION 1..8: note = source = /note="Description of Artificial Sequence: Syntheticpeptide"
GFTFDDYA

SEQ ID NO: 37 - protein, 8 aa, synthetic construct
  REGION 1..8: note = source = /note="Description of Artificial Sequence: Syntheticpeptide"
ISWNSGSI

SEQ ID NO: 38 - protein, 16 aa, synthetic construct
  REGION 1..16: note = source = /note="Description of Artificial Sequence: Syntheticpeptide"
AKDSRGYGDYRLGGAY

SEQ ID NO: 39 - protein, 6 aa, synthetic construct
  REGION 1..6: note = source = /note="Description of Artificial Sequence: Syntheticpeptide"
QSVSSN

SEQ ID NO: 40 - skipped

SEQ ID NO: 41 - protein, 9 aa, synthetic construct
  REGION 1..9: note = source = /note="Description of Artificial Sequence: Syntheticpeptide"
QQYNNWPWT

SEQ ID NO: 42 - protein, 123 aa, synthetic construct
  REGION 1..123: note = source = /note="Description of Artificial Sequence: Syntheticpolypeptide"
EVQLVESGGGLVQPGRSLRLSCAASGFTFDDYAMHWVRQAPGKGLEWVSGISWNSGSIGYADSVKGRFTISRDNAKNSLYLQMNSLRAEDTALYYCAKDSRGYGDYRLGGAYWGQGTLVTVSS

SEQ ID NO: 43 - protein, 107 aa, synthetic construct
  REGION 1..107: note = source = /note="Description of Artificial Sequence: Syntheticpolypeptide"
EIVMTQSPATLSVSPGERATLSCRASQSVSSNLAWYQQKPGQAPRLLIYGASTRATGIPARFSGSGSGTEFTLTISSLQSEDFAVYYCQQYNNWPWTFGQGTKVEIK

SEQ ID NO: 44 - protein, 329 aa, Homo sapiens
ASTKGPSVFPLAPSSKSTSGGTAALGCLVKDYFPEPVTVSWNSGALTSGVHTFPAVLQSSGLYSLSSVVTVPSSSLGTQTYICNVNHKPSNTKVDKKVEPKSCDKTHTCPPCPAPELLGGPSVFLFPPKPKDTLMISRTPEVTCVVVDVSHEDPEVKFNWYVDGVEVHNAKTKPREEQYNSTYRVVSVLTVLHQDWLNGKEYKCKVSNKALPAPIEKTISKAKGQPREPQVYTLPPSDELTKNQVSLTCLVKGFYPSDIAVEWESNGQPENNYKTTPPVLDSDGSFFLYSKLTVDKSRWQQGNVFSCSVMHEALHNHYTQKSLSLSPGK

SEQ ID NO: 45 - protein, 327 aa, Homo sapiens
ASTKGPSVFPLAPCSRSTSESTAALGCLVKDYFPEPVTVSWNSGALTSGVHTFPAVLQSSGLYSLSSVVTVPSSSLGTKTYTCNVDHKPSNTKVDKRVESKYGPPCPSCPAPEFLGGPSVFLFPPKPKDTLMISRTPEVTCVVVDVSQEDPEVQFNWYVDGVEVHNAKTKPREEQFNSTYRVVSVLTVLHQDWLNGKEYKCKVSNKGLPSSIEKTISKAKGQPREPQVYTLPPSQEEMTKNQVSLTCLVKGFYPSDIAVEWESNGQPENNYKTTPPVLDSDGSFFLYSRLTVDKSRWQEGNVFSCSVMHEALHNHYTQKSLSLSLGK

SEQ ID NO: 46 - protein, 330 aa, synthetic construct
  REGION 1..330: note = source = /note="Description of Artificial Sequence: Syntheticpolypeptide"
ASTKGPSVFPLAPSSKSTSGGTAALGCLVKDYFPEPVTVSWNSGALTSGVHTFPAVLQSSGLYSLSSVVTVPSSSLGTQTYICNVNHKPSNTKVDKKVEPKSCDKTHTCPPCPAPEAAGGPSVFLFPPKPKDTLMISRTPEVTCVVVDVSHEDPEVKFNWYVDGVEVHNAKTKPREEQYNSTYRVVSVLTVLHQDWLNGKEYKCKVSNKALPAPIEKTISKAKGQPREPQVYTLPPSREEMTKNQVSLTCLVKGFYPSDIAVEWESNGQPENNYKTTPPVLDSDGSFFLYSKLTVDKSRWQQGNVFSCSVMHEALHNHYTQKSLSLSPGK

SEQ ID NO: 47 - protein, 327 aa, synthetic construct
  REGION 1..327: note = source = /note="Description of Artificial Sequence: Syntheticpolypeptide"
ASTKGPSVFPLAPCSRSTSESTAALGCLVKDYFPEPVTVSWNSGALTSGVHTFPAVLQSSGLYSLSSVVTVPSSSLGTKTYTCNVDHKPSNTKVDKRVESKYGPPCPPCPAPEAAGGPSVFLFPPKPKDTLMISRTPEVTCVVVDVSQEDPEVQFNWYVDGVEVHNAKTKPREEQFNSTYRVVSVLTVLHQDWLNGKEYKCKVSNKGLPSSIEKTISKAKGQPREPQVYTLPPSQEEMTKNQVSLTCLVKGFYPSDIAVEWESNGQPENNYKTTPPVLDSDGSFFLYSRLTVDKSRWQEGNVFSCSVMHEALHNHYTQKSLSLSLGK

SEQ ID NO: 48 - protein, 107 aa, synthetic construct [sequence omitted]

SEQ ID NO: 49 - protein, 214 aa, synthetic construct
  REGION 1..214: note = source = /note="Description of Artificial Sequence: Syntheticpolypeptide"
EIVMTQSPATLSVSPGERATLSCRASQSVSSNLAWYQQKPGQAPRLLIYGASTRATGIPARFSGSGSGTEFTLTISSLQSEDFAVYYCQQYNNWPWTFGQGTKVEIKRTVAAPSVFIFPPSDEQLKSGTASVVCLLNNFYPREAKVQWKVDNALQSGNSQESVTEQDSKDSTYSLSSTLTLSKADYEKHKVYACEVTHQGLSSPVTKSFNRGEC

SEQ ID NO: 50 - protein, 453 aa, synthetic construct
  REGION 1..453: note = source = /note="Description of Artificial Sequence: Syntheticpolypeptide"
EVQLVESGGGLVQPGRSLRLSCAASGFTFDDYAMHWVRQAPGKGLEWVSGISWNSGSIGYADSVKGRFTISRDNAKNSLYLQMNSLRAEDTALYYCAKDSRGYGDYRLGGAYWGQGTLVTVSSASTKGPSVFPLAPSSKSTSGGTAALGCLVKDYFPEPVTVSWNSGALTSGVHTFPAVLQSSGLYSLSSVVTVPSSSLGTQTYICNVNHKPSNTKVDKKVEPKSCDKTHTCPPCPAPELLGGPSVFLFPPKPKDTLMISRTPEVTCVVVDVSHEDPEVKFNWYVDGVEVHNAKTKPREEQYNSTYRVVSVLTVLHQDWLNGKEYKCKVSNKALPAPIEKTISKAKGQPREPQVYTLPPSREEMTKNQVSLTCLVKGFYPSDIAVEWESNGQPENNYKTTPPVLDSDGSFFLYSKLTVDKSRWQQGNVFSCSVMHEALHNHYTQKSLSLSPGK

SEQ ID NO: 51 - protein, 453 aa, synthetic construct
  REGION 1..453: note = source = /note="Description of Artificial Sequence: Syntheticpolypeptide"
EVQLVESGGGLVQPGRSLRLSCAASGFTFDDYAMHWVRQAPGKGLEWVSGISWNSGSIGYADSVKGRFTISRDNAKNSLYLQMNSLRAEDTALYYCAKDSRGYGDYRLGGAYWGQGTLVTVSSASTKGPSVFPLAPSSKSTSGGTAALGCLVKDYFPEPVTVSWNSGALTSGVHTFPAVLQSSGLYSLSSVVTVPSSSLGTQTYICNVNHKPSNTKVDKKVEPKSCDKTHTCPPCPAPEAAGGPSVFLFPPKPKDTLMISRTPEVTCVVVDVSHEDPEVKFNWYVDGVEVHNAKTKPREEQYNSTYRVVSVLTVLHQDWLNGKEYKCKVSNKALPAPIEKTISKAKGQPREPQVYTLPPSREEMTKNQVSLTCLVKGFYPSDIAVEWESNGQPENNYKTTPPVLDSDGSFFLYSKLTVDKSRWQQGNVFSCSVMHEALHNHYTQKSLSLSPGK

SEQ ID NO: 52 - protein, 450 aa, synthetic construct
  REGION 1..450: note = source = /note="Description of Artificial Sequence: Syntheticpolypeptide"
EVQLVESGGGLVQPGRSLRLSCAASGFTFDDYAMHWVRQAPGKGLEWVSGISWNSGSIGYADSVKGRFTISRDNAKNSLYLQMNSLRAEDTALYYCAKDSRGYGDYRLGGAYWGQGTLVTVSSASTKGPSVFPLAPCSRSTSESTAALGCLVKDYFPEPVTVSWNSGALTSGVHTFPAVLQSSGLYSLSSVVTVPSSSLGTKTYTCNVDHKPSNTKVDKRVESKYGPPCPSCPAPEFLGGPSVFLFPPKPKDTLMISRTPEVTCVVVDVSQEDPEVQFNWYVDGVEVHNAKTKPREEQFNSTYRVVSVLTVLHQDWLNGKEYKCKVSNKGLPSSIEKTISKAKGQPREPQVYTLPPSQEEMTKNQVSLTCLVKGFYPSDIAVEWESNGQPENNYKTTPPVLDSDGSFFLYSRLTVDKSRWQEGNVFSCSVMHEALHNHYTQKSLSLSLGK

SEQ ID NO: 53 - protein, 450 aa, synthetic construct
  REGION 1..450: note = source = /note="Description of Artificial Sequence: Syntheticpolypeptide"
EVQLVESGGGLVQPGRSLRLSCAASGFTFDDYAMHWVRQAPGKGLEWVSGISWNSGSIGYADSVKGRFTISRDNAKNSLYLQMNSLRAEDTALYYCAKDSRGYGDYRLGGAYWGQGTLVTVSSASTKGPSVFPLAPCSRSTSESTAALGCLVKDYFPEPVTVSWNSGALTSGVHTFPAVLQSSGLYSLSSVVTVPSSSLGTKTYTCNVDHKPSNTKVDKRVESKYGPPCPPCPAPEAAGGPSVFLFPPKPKDTLMISRTPEVTCVVVDVSQEDPEVQFNWYVDGVEVHNAKTKPREEQFNSTYRVVSVLTVLHQDWLNGKEYKCKVSNKGLPSSIEKTISKAKGQPREPQVYTLPPSQEEMTKNQVSLTCLVKGFYPSDIAVEWESNGQPENNYKTTPPVLDSDGSFFLYSRLTVDKSRWQEGNVFSCSVMHEALHNHYTQKSLSLSLGK

SEQ ID NO: 54 - protein, 229 aa, synthetic construct
  REGION 1..229: note = source = /note="Description of Artificial Sequence: Syntheticpolypeptide"
ESKYGPPCPPCPAPEAAGGPSVFLFPPKPKDTLMISRTPEVTCVVVDVSQEDPEVQFNWYVDGVEVHNAKTKPREEQFNSTYRVVSVLTVLHQDWLNGKEYKCKVSNKGLPSSIEKTISKAKGQPREPQVYTLPPSQEEMTKNQVSLSCAVKGFYPSDIAVEWESNGQPENNYKTTPPVLDSDGSFFLVSRLTVDKSRWQEGNVFSCSVMHEALHNHYTQKSLSLSLGK

SEQ ID NO: 55 - protein, 229 aa, synthetic construct
  REGION 1..229: note = source = /note="Description of Artificial Sequence: Syntheticpolypeptide"
ESKYGPPCPPCPAPEAAGGPSVFLFPPKPKDTLMISRTPEVTCVVVDVSQEDPEVQFNWYVDGVEVHNAKTKPREEQFNSTYRVVSVLTVLHQDWLNGKEYKCKVSNKGLPSSIEKTISKAKGQPREPQVYTLPPSQEEMTKNQVSLWCLVKGFYPSDIAVEWESNGQPENNYKTTPPVLDSDGSFFLYSRLTVDKSRWQEGNVFSCSVMHEALHNHYTQKSLSLSLGK

SEQ ID NO: 56 - protein, 450 aa, synthetic construct
  REGION 1..450: note = source = /note="Description of Artificial Sequence: Syntheticpolypeptide"
EVQLVESGGGLVQPGRSLRLSCAASGFTFDDYAMHWVRQAPGKGLEWVSGISWNSGSIGYADSVKGRFTISRDNAKNSLYLQMNSLRAEDTALYYCAKDSRGYGDYRLGGAYWGQGTLVTVSSASTKGPSVFPLAPCSRSTSESTAALGCLVKDYFPEPVTVSWNSGALTSGVHTFPAVLQSSGLYSLSSVVTVPSSSLGTKTYTCNVDHKPSNTKVDKRVESKYGPPCPPCPAPEAAGGPSVFLFPPKPKDTLMISRTPEVTCVVVDVSQEDPEVQFNWYVDGVEVHNAKTKPREEQFNSTYRVVSVLTVLHQDWLNGKEYKCKVSNKGLPSSIEKTISKAKGQPREPQVYTLPPSQEEMTKNQVSLWCLVKGFYPSDIAVEWESNGQPENNYKTTPPVLDSDGSFFLYSRLTVDKSRWQEGNVFSCSVMHEALHNHYTQKSLSLSLGK

SEQ ID NO: 57 - protein, 450 aa, synthetic construct
  REGION 1..450: note = source = /note="Description of Artificial Sequence: Syntheticpolypeptide"
EVQLVESGGGLVQPGRSLRLSCAASGFTFDDYAMHWVRQAPGKGLEWVSGISWNSGSIGYADSVKGRFTISRDNAKNSLYLQMNSLRAEDTALYYCAKDSRGYGDYRLGGAYWGQGTLVTVSSASTKGPSVFPLAPCSRSTSESTAALGCLVKDYFPEPVTVSWNSGALTSGVHTFPAVLQSSGLYSLSSVVTVPSSSLGTKTYTCNVDHKPSNTKVDKRVESKYGPPCPPCPAPEAAGGPSVFLFPPKPKDTLMISRTPEVTCVVVDVSQEDPEVQFNWYVDGVEVHNAKTKPREEQFNSTYRVVSVLTVLHQDWLNGKEYKCKVSNKGLPSSIEKTISKAKGQPREPQVYTLPPSQEEMTKNQVSLSCAVKGFYPSDIAVEWESNGQPENNYKTTPPVLDSDGSFFLVSRLTVDKSRWQEGNVFSCSVMHEALHNHYTQKSLSLSLGK

SEQ ID NO: 58 - protein, 472 aa, synthetic construct
  REGION 1..472: note = source = /note="Description of Artificial Sequence: Syntheticpolypeptide"
EVQLLESGGGLVQPGGSLRLSCAASGFTVSSYGMSWVRQAPGKGPEWVSGIRGSDGSTYYADSVKGRFTISRDNSKNTLYLQMNSLRAEDTAVYYCAKQGENDGPFDHRGQGTLVTVSSGGGGSEVQLLESGGGLVQPGGSLRLSCAASGFTVSSYGMSWVRQAPGKGPEWVSGIRGSDGSTYYADSVKGRFTISRDNSKNTLYLQMNSLRAEDTAVYYCAKQGENDGPFDHRGQGTLVTVSSESKYGPPCPPCPAPEAAGGPSVFLFPPKPKDTLMISRTPEVTCVVVDVSQEDPEVQFNWYVDGVEVHNAKTKPREEQFNSTYRVVSVLTVLHQDWLNGKEYKCKVSNKGLPSSIEKTISKAKGQPREPQVYTLPPSQEEMTKNQVSLSCAVKGFYPSDIAVEWESNGQPENNYKTTPPVLDSDGSFFLVSRLTVDKSRWQEGNVFSCSVMHEALHNHYTQKSLSLSLGK

SEQ ID NO: 59 - protein, 477 aa, synthetic construct
  REGION 1..477: note = source = /note="Description of Artificial Sequence: Syntheticpolypeptide"
EVQLLESGGGLVQPGGSLRLSCAASGFTVSSYGMSWVRQAPGKGPEWVSGIRGSDGSTYYADSVKGRFTISRDNSKNTLYLQMNSLRAEDTAVYYCAKQGENDGPFDHRGQGTLVTVSSGGGGSGGGGSEVQLLESGGGLVQPGGSLRLSCAASGFTVSSYGMSWVRQAPGKGPEWVSGIRGSDGSTYYADSVKGRFTISRDNSKNTLYLQMNSLRAEDTAVYYCAKQGENDGPFDHRGQGTLVTVSSESKYGPPCPPCPAPEAAGGPSVFLFPPKPKDTLMISRTPEVTCVVVDVSQEDPEVQFNWYVDGVEVHNAKTKPREEQFNSTYRVVSVLTVLHQDWLNGKEYKCKVSNKGLPSSIEKTISKAKGQPREPQVYTLPPSQEEMTKNQVSLSCAVKGFYPSDIAVEWESNGQPENNYKTTPPVLDSDGSFFLVSRLTVDKSRWQEGNVFSCSVMHEALHNHYTQKSLSLSLGK

SEQ ID NO: 60 - protein, 348 aa, synthetic construct
  REGION 1..348: note = source = /note="Description of Artificial Sequence: Syntheticpolypeptide"
EVQLLESGGGLVQPGGSLRLSCAASGFTVSSYGMSWVRQAPGKGPEWVSGIRGSDGSTYYADSVKGRFTISRDNSKNTLYLQMNSLRAEDTAVYYCAKQGENDGPFDHRGQGTLVTVSSESKYGPPCPPCPAPEAAGGPSVFLFPPKPKDTLMISRTPEVTCVVVDVSQEDPEVQFNWYVDGVEVHNAKTKPREEQFNSTYRVVSVLTVLHQDWLNGKEYKCKVSNKGLPSSIEKTISKAKGQPREPQVYTLPPSQEEMTKNQVSLSCAVKGFYPSDIAVEWESNGQPENNYKTTPPVLDSDGSFFLVSRLTVDKSRWQEGNVFSCSVMHEALHNHYTQKSLSLSLGK

SEQ ID NO: 61 - protein, 349 aa, synthetic construct
  REGION 1..349: note = source = /note="Description of Artificial Sequence: Syntheticpolypeptide"
QLQLQESGPGLVKPSETLSLTCTVSGGSISSSNYFWGWIRQSPGKGLEWIGSIDYSGYTYYNPSLKSRVTISVDTSKNQFSLKLSSVTAADTAVYNCARHKAATADFDYRGQGTLVTVSSESKYGPPCPPCPAPEAAGGPSVFLFPPKPKDTLMISRTPEVTCVVVDVSQEDPEVQFNWYVDGVEVHNAKTKPREEQFNSTYRVVSVLTVLHQDWLNGKEYKCKVSNKGLPSSIEKTISKAKGQPREPQVYTLPPSQEEMTKNQVSLSCAVKGFYPSDIAVEWESNGQPENNYKTTPPVLDSDGSFFLVSRLTVDKSRWQEGNVFSCSVMHEALHNHYTQKSLSLSLGK

SEQ ID NO: 62 - protein, 479 aa, synthetic construct
  REGION 1..479: note = source = /note="Description of Artificial Sequence: Syntheticpolypeptide"
QLQLQESGPGLVKPSETLSLTCTVSGGSISSSNYFWGWIRQSPGKGLEWIGSIDYSGYTYYNPSLKSRVTISVDTSKNQFSLKLSSVTAADTAVYNCARHKAATADFDYRGQGTLVTVSSGGGGSGGGGSQLQLQESGPGLVKPSETLSLTCTVSGGSISSSNYFWGWIRQSPGKGLEWIGSIDYSGYTYYNPSLKSRVTISVDTSKNQFSLKLSSVTAADTAVYNCARHKAATADFDYRGQGTLVTVSSESKYGPPCPPCPAPEAAGGPSVFLFPPKPKDTLMISRTPEVTCVVVDVSQEDPEVQFNWYVDGVEVHNAKTKPREEQFNSTYRVVSVLTVLHQDWLNGKEYKCKVSNKGLPSSIEKTISKAKGQPREPQVYTLPPSQEEMTKNQVSLSCAVKGFYPSDIAVEWESNGQPENNYKTTPPVLDSDGSFFLVSRLTVDKSRWQEGNVFSCSVMHEALHNHYTQKSLSLSLGK

SEQ ID NO: 63 - protein, 356 aa, synthetic construct
  REGION 1..356: note = source = /note="Description of Artificial Sequence: Syntheticpolypeptide"
QVQLVESGGGVVQPGRSLRLSCAASGFSFSRYGMHWVRQAPGKGLEGVAVIWYDGSNRYYADSVKGRFTISRDNSKNTLYLQMNSLRAEDTAVYYCAREPRIGYYYESSGYYSLDYRGQGTLVTVSSESKYGPPCPPCPAPEAAGGPSVFLFPPKPKDTLMISRTPEVTCVVVDVSQEDPEVQFNWYVDGVEVHNAKTKPREEQFNSTYRVVSVLTVLHQDWLNGKEYKCKVSNKGLPSSIEKTISKAKGQPREPQVYTLPPSQEEMTKNQVSLSCAVKGFYPSDIAVEWESNGQPENNYKTTPPVLDSDGSFFLVSRLTVDKSRWQEGNVFSCSVMHEALHNHYTQKSLSLSLGK

SEQ ID NO: 64 - protein, 493 aa, synthetic construct
  REGION 1..493: note = source = /note="Description of Artificial Sequence: Syntheticpolypeptide"
QVQLVESGGGVVQPGRSLRLSCAASGFSFSRYGMHWVRQAPGKGLEGVAVIWYDGSNRYYADSVKGRFTISRDNSKNTLYLQMNSLRAEDTAVYYCAREPRIGYYYESSGYYSLDYRGQGTLVTVSSGGGGSGGGGSQVQLVESGGGVVQPGRSLRLSCAASGFSFSRYGMHWVRQAPGKGLEGVAVIWYDGSNRYYADSVKGRFTISRDNSKNTLYLQMNSLRAEDTAVYYCAREPRIGYYYESSGYYSLDYRGQGTLVTVSSESKYGPPCPPCPAPEAAGGPSVFLFPPKPKDTLMISRTPEVTCVVVDVSQEDPEVQFNWYVDGVEVHNAKTKPREEQFNSTYRVVSVLTVLHQDWLNGKEYKCKVSNKGLPSSIEKTISKAKGQPREPQVYTLPPSQEEMTKNQVSLSCAVKGFYPSDIAVEWESNGQPENNYKTTPPVLDSDGSFFLVSRLTVDKSRWQEGNVFSCSVMHEALHNHYTQKSLSLSLGK

SEQ ID NO: 65 - protein, 486 aa, synthetic construct
  REGION 1..486: note = source = /note="Description of Artificial Sequence: Syntheticpolypeptide"
QLQLQESGPGLVKPSETLSLTCTVSGGSISSSNYFWGWIRQSPGKGLEWIGSIDYSGYTYYNPSLKSRVTISVDTSKNQFSLKLSSVTAADTAVYNCARHKAATADFDYRGQGTLVTVSSGGGGSGGGGSQVQLVESGGGVVQPGRSLRLSCAASGFSFSRYGMHWVRQAPGKGLEGVAVIWYDGSNRYYADSVKGRFTISRDNSKNTLYLQMNSLRAEDTAVYYCAREPRIGYYYESSGYYSLDYRGQGTLVTVSSESKYGPPCPPCPAPEAAGGPSVFLFPPKPKDTLMISRTPEVTCVVVDVSQEDPEVQFNWYVDGVEVHNAKTKPREEQFNSTYRVVSVLTVLHQDWLNGKEYKCKVSNKGLPSSIEKTISKAKGQPREPQVYTLPPSQEEMTKNQVSLSCAVKGFYPSDIAVEWESNGQPENNYKTTPPVLDSDGSFFLVSRLTVDKSRWQEGNVFSCSVMHEALHNHYTQKSLSLSLGK

SEQ ID NO: 66 - protein, 486 aa, synthetic construct
  REGION 1..486: note = source = /note="Description of Artificial Sequence: Syntheticpolypeptide"
QVQLVESGGGVVQPGRSLRLSCAASGFSFSRYGMHWVRQAPGKGLEGVAVIWYDGSNRYYADSVKGRFTISRDNSKNTLYLQMNSLRAEDTAVYYCAREPRIGYYYESSGYYSLDYRGQGTLVTVSSGGGGSGGGGSQLQLQESGPGLVKPSETLSLTCTVSGGSISSSNYFWGWIRQSPGKGLEWIGSIDYSGYTYYNPSLKSRVTISVDTSKNQFSLKLSSVTAADTAVYNCARHKAATADFDYRGQGTLVTVSSESKYGPPCPPCPAPEAAGGPSVFLFPPKPKDTLMISRTPEVTCVVVDVSQEDPEVQFNWYVDGVEVHNAKTKPREEQFNSTYRVVSVLTVLHQDWLNGKEYKCKVSNKGLPSSIEKTISKAKGQPREPQVYTLPPSQEEMTKNQVSLSCAVKGFYPSDIAVEWESNGQPENNYKTTPPVLDSDGSFFLVSRLTVDKSRWQEGNVFSCSVMHEALHNHYTQKSLSLSLGK

SEQ ID NO: 67 - protein, 345 aa, synthetic construct
  REGION 1..345: note = source = /note="Description of Artificial Sequence: Syntheticpolypeptide"
EVQLVESGGGLVQPGGSLRLSCAASGFSFSDFWMSWVRQAPGKGLEWVATISQAGSEKDYVDSVKGRFTISRDNAKKSLYLQMNSLRAEDTAVYYCASGVYSFDYRGQGTLVTVSSESKYGPPCPPCPAPEAAGGPSVFLFPPKPKDTLMISRTPEVTCVVVDVSQEDPEVQFNWYVDGVEVHNAKTKPREEQFNSTYRVVSVLTVLHQDWLNGKEYKCKVSNKGLPSSIEKTISKAKGQPREPQVYTLPPSQEEMTKNQVSLSCAVKGFYPSDIAVEWESNGQPENNYKTTPPVLDSDGSFFLVSRLTVDKSRWQEGNVFSCSVMHEALHNHYTQKSLSLSLGK

SEQ ID NO: 68 - protein, 466 aa, synthetic construct
  REGION 1..466: note = source = /note="Description of Artificial Sequence: Syntheticpolypeptide"
EVQLVESGGGLVQPGGSLRLSCAASGFSFSDFWMSWVRQAPGKGLEWVATISQAGSEKDYVDSVKGRFTISRDNAKKSLYLQMNSLRAEDTAVYYCASGVYSFDYRGQGTLVTVSSGGGGSEVQLVESGGGLVQPGGSLRLSCAASGFSFSDFWMSWVRQAPGKGLEWVATISQAGSEKDYVDSVKGRFTISRDNAKKSLYLQMNSLRAEDTAVYYCASGVYSFDYRGQGTLVTVSSESKYGPPCPPCPAPEAAGGPSVFLFPPKPKDTLMISRTPEVTCVVVDVSQEDPEVQFNWYVDGVEVHNAKTKPREEQFNSTYRVVSVLTVLHQDWLNGKEYKCKVSNKGLPSSIEKTISKAKGQPREPQVYTLPPSQEEMTKNQVSLSCAVKGFYPSDIAVEWESNGQPENNYKTTPPVLDSDGSFFLVSRLTVDKSRWQEGNVFSCSVMHEALHNHYTQKSLSLSLGK

SEQ ID NO: 69 - protein, 471 aa, synthetic construct
  REGION 1..471: note = source = /note="Description of Artificial Sequence: Syntheticpolypeptide"
EVQLVESGGGLVQPGGSLRLSCAASGFSFSDFWMSWVRQAPGKGLEWVATISQAGSEKDYVDSVKGRFTISRDNAKKSLYLQMNSLRAEDTAVYYCASGVYSFDYRGQGTLVTVSSGGGGSGGGGSEVQLVESGGGLVQPGGSLRLSCAASGFSFSDFWMSWVRQAPGKGLEWVATISQAGSEKDYVDSVKGRFTISRDNAKKSLYLQMNSLRAEDTAVYYCASGVYSFDYRGQGTLVTVSSESKYGPPCPPCPAPEAAGGPSVFLFPPKPKDTLMISRTPEVTCVVVDVSQEDPEVQFNWYVDGVEVHNAKTKPREEQFNSTYRVVSVLTVLHQDWLNGKEYKCKVSNKGLPSSIEKTISKAKGQPREPQVYTLPPSQEEMTKNQVSLSCAVKGFYPSDIAVEWESNGQPENNYKTTPPVLDSDGSFFLVSRLTVDKSRWQEGNVFSCSVMHEALHNHYTQKSLSLSLGK

SEQ ID NO: 70 - protein, 5 aa, synthetic construct
  REGION 1..5: note = source = /note="Description of Artificial Sequence: Syntheticpeptide"
GGGGS

SEQ ID NO: 71 - protein, 10 aa, synthetic construct
  REGION 1..10: note = source = /note="Description of Artificial Sequence: Syntheticpeptide"
GGGGSGGGGS

SEQ ID NO: 72 - protein, 327 aa, synthetic construct
  REGION 1..327: note = source = /note="Description of Artificial Sequence: Syntheticpolypeptide"
ASTKGPSVFPLAPCSRSTSESTAALGCLVKDYFPEPVTVSWNSGALTSGVHTFPAVLQSSGLYSLSSVVTVPSSSLGTKTYTCNVDHKPSNTKVDKRVESKYGPPCPPCPAPEAAGGPSVFLFPPKPKDTLMISRTPEVTCVVVDVSQEDPEVQFNWYVDGVEVHNAKTKPREEQFNSTYRVVSVLTVLHQDWLNGKEYKCKVSNKGLPSSIEKTISKAKGQPREPQVYTLPPSQEEMTKNQVSLSCAVKGFYPSDIAVEWESNGQPENNYKTTPPVLDSDGSFFLVSRLTVDKSRWQEGNVFSCSVMHEALHNHYTQKSLSLSLGK

SEQ ID NO: 73 - protein, 327 aa, synthetic construct
  REGION 1..327: note = source = /note="Description of Artificial Sequence: Syntheticpolypeptide"
ASTKGPSVFPLAPCSRSTSESTAALGCLVKDYFPEPVTVSWNSGALTSGVHTFPAVLQSSGLYSLSSVVTVPSSSLGTKTYTCNVDHKPSNTKVDKRVESKYGPPCPPCPAPEAAGGPSVFLFPPKPKDTLMISRTPEVTCVVVDVSQEDPEVQFNWYVDGVEVHNAKTKPREEQFNSTYRVVSVLTVLHQDWLNGKEYKCKVSNKGLPSSIEKTISKAKGQPREPQVYTLPPSQEEMTKNQVSLWCLVKGFYPSDIAVEWESNGQPENNYKTTPPVLDSDGSFFLYSRLTVDKSRWQEGNVFSCSVMHEALHNHYTQKSLSLSLGK

SEQ ID NO: 74 - skipped

SEQ ID NO: 75 - protein, 449 aa, synthetic construct
  REGION 1..449: note = source = /note="Description of Artificial Sequence: Syntheticpolypeptide"
EVQLVESGGGLVQPGRSLRLSCAASGFTFDDYAMHWVRQAPGKGLEWVSGISWNSGSIGYADSVKGRFTISRDNAKNSLYLQMNSLRAEDTALYYCAKDSRGYGDYRLGGAYWGQGTLVTVSSASTKGPSVFPLAPCSRSTSESTAALGCLVKDYFPEPVTVSWNSGALTSGVHTFPAVLQSSGLYSLSSVVTVPSSSLGTKTYTCNVDHKPSNTKVDKRVESKYGPPCPPCPAPEAAGGPSVFLFPPKPKDTLMISRTPEVTCVVVDVSQEDPEVQFNWYVDGVEVHNAKTKPREEQFNSTYRVVSVLTVLHQDWLNGKEYKCKVSNKGLPSSIEKTISKAKGQPREPQVYTLPPSQEEMTKNQVSLWCLVKGFYPSDIAVEWESNGQPENNYKTTPPVLDSDGSFFLYSRLTVDKSRWQEGNVFSCSVMHEALHNHYTQKSLSLSLG

SEQ ID NO: 76 - protein, 471 aa, synthetic construct
  REGION 1..471: note = source = /note="Description of Artificial Sequence: Syntheticpolypeptide"
EVQLLESGGGLVQPGGSLRLSCAASGFTVSSYGMSWVRQAPGKGPEWVSGIRGSDGSTYYADSVKGRFTISRDNSKNTLYLQMNSLRAEDTAVYYCAKQGENDGPFDHRGQGTLVTVSSGGGGSEVQLLESGGGLVQPGGSLRLSCAASGFTVSSYGMSWVRQAPGKGPEWVSGIRGSDGSTYYADSVKGRFTISRDNSKNTLYLQMNSLRAEDTAVYYCAKQGENDGPFDHRGQGTLVTVSSESKYGPPCPPCPAPEAAGGPSVFLFPPKPKDTLMISRTPEVTCVVVDVSQEDPEVQFNWYVDGVEVHNAKTKPREEQFNSTYRVVSVLTVLHQDWLNGKEYKCKVSNKGLPSSIEKTISKAKGQPREPQVYTLPPSQEEMTKNQVSLSCAVKGFYPSDIAVEWESNGQPENNYKTTPPVLDSDGSFFLVSRLTVDKSRWQEGNVFSCSVMHEALHNHYTQKSLSLSLG

SEQ ID NO: 77 - protein, 476 aa, synthetic construct
  REGION 1..476: note = source = /note="Description of Artificial Sequence: Syntheticpolypeptide"
EVQLLESGGGLVQPGGSLRLSCAASGFTVSSYGMSWVRQAPGKGPEWVSGIRGSDGSTYYADSVKGRFTISRDNSKNTLYLQMNSLRAEDTAVYYCAKQGENDGPFDHRGQGTLVTVSSGGGGSGGGGSEVQLLESGGGLVQPGGSLRLSCAASGFTVSSYGMSWVRQAPGKGPEWVSGIRGSDGSTYYADSVKGRFTISRDNSKNTLYLQMNSLRAEDTAVYYCAKQGENDGPFDHRGQGTLVTVSSESKYGPPCPPCPAPEAAGGPSVFLFPPKPKDTLMISRTPEVTCVVVDVSQEDPEVQFNWYVDGVEVHNAKTKPREEQFNSTYRVVSVLTVLHQDWLNGKEYKCKVSNKGLPSSIEKTISKAKGQPREPQVYTLPPSQEEMTKNQVSLSCAVKGFYPSDIAVEWESNGQPENNYKTTPPVLDSDGSFFLVSRLTVDKSRWQEGNVFSCSVMHEALHNHYTQKSLSLSLG

SEQ ID NO: 78 - protein, 344 aa, synthetic construct
  REGION 1..344: note = source = /note="Description of Artificial Sequence: Syntheticpolypeptide"
EVQLVESGGGLVQPGGSLRLSCAASGFSFSDFWMSWVRQAPGKGLEWVATISQAGSEKDYVDSVKGRFTISRDNAKKSLYLQMNSLRAEDTAVYYCASGVYSFDYRGQGTLVTVSSESKYGPPCPPCPAPEAAGGPSVFLFPPKPKDTLMISRTPEVTCVVVDVSQEDPEVQFNWYVDGVEVHNAKTKPREEQFNSTYRVVSVLTVLHQDWLNGKEYKCKVSNKGLPSSIEKTISKAKGQPREPQVYTLPPSQEEMTKNQVSLSCAVKGFYPSDIAVEWESNGQPENNYKTTPPVLDSDGSFFLVSRLTVDKSRWQEGNVFSCSVMHEALHNHYTQKSLSLSLG

SEQ ID NO: 79 - protein, 465 aa, synthetic construct
  REGION 1..465: note = source = /note="Description of Artificial Sequence: Syntheticpolypeptide"
EVQLVESGGGLVQPGGSLRLSCAASGFSFSDFWMSWVRQAPGKGLEWVATISQAGSEKDYVDSVKGRFTISRDNAKKSLYLQMNSLRAEDTAVYYCASGVYSFDYRGQGTLVTVSSGGGGSEVQLVESGGGLVQPGGSLRLSCAASGFSFSDFWMSWVRQAPGKGLEWVATISQAGSEKDYVDSVKGRFTISRDNAKKSLYLQMNSLRAEDTAVYYCASGVYSFDYRGQGTLVTVSSESKYGPPCPPCPAPEAAGGPSVFLFPPKPKDTLMISRTPEVTCVVVDVSQEDPEVQFNWYVDGVEVHNAKTKPREEQFNSTYRVVSVLTVLHQDWLNGKEYKCKVSNKGLPSSIEKTISKAKGQPREPQVYTLPPSQEEMTKNQVSLSCAVKGFYPSDIAVEWESNGQPENNYKTTPPVLDSDGSFFLVSRLTVDKSRWQEGNVFSCSVMHEALHNHYTQKSLSLSLG

SEQ ID NO: 80 - protein, 470 aa, synthetic construct
  REGION 1..470: note = source = /note="Description of Artificial Sequence: Syntheticpolypeptide"
EVQLVESGGGLVQPGGSLRLSCAASGFSFSDFWMSWVRQAPGKGLEWVATISQAGSEKDYVDSVKGRFTISRDNAKKSLYLQMNSLRAEDTAVYYCASGVYSFDYRGQGTLVTVSSGGGGSGGGGSEVQLVESGGGLVQPGGSLRLSCAASGFSFSDFWMSWVRQAPGKGLEWVATISQAGSEKDYVDSVKGRFTISRDNAKKSLYLQMNSLRAEDTAVYYCASGVYSFDYRGQGTLVTVSSESKYGPPCPPCPAPEAAGGPSVFLFPPKPKDTLMISRTPEVTCVVVDVSQEDPEVQFNWYVDGVEVHNAKTKPREEQFNSTYRVVSVLTVLHQDWLNGKEYKCKVSNKGLPSSIEKTISKAKGQPREPQVYTLPPSQEEMTKNQVSLSCAVKGFYPSDIAVEWESNGQPENNYKTTPPVLDSDGSFFLVSRLTVDKSRWQEGNVFSCSVMHEALHNHYTQKSLSLSLG

SEQ ID NO: 81 - protein, 348 aa, synthetic construct
  REGION 1..348: note = source = /note="Description of Artificial Sequence: Syntheticpolypeptide"
QLQLQESGPGLVKPSETLSLTCTVSGGSISSSNYFWGWIRQSPGKGLEWIGSIDYSGYTYYNPSLKSRVTISVDTSKNQFSLKLSSVTAADTAVYNCARHKAATADFDYRGQGTLVTVSSESKYGPPCPPCPAPEAAGGPSVFLFPPKPKDTLMISRTPEVTCVVVDVSQEDPEVQFNWYVDGVEVHNAKTKPREEQFNSTYRVVSVLTVLHQDWLNGKEYKCKVSNKGLPSSIEKTISKAKGQPREPQVYTLPPSQEEMTKNQVSLSCAVKGFYPSDIAVEWESNGQPENNYKTTPPVLDSDGSFFLVSRLTVDKSRWQEGNVFSCSVMHEALHNHYTQKSLSLSLG

SEQ ID NO: 82 - protein, 478 aa, synthetic construct
  REGION 1..478: note = source = /note="Description of Artificial Sequence: Syntheticpolypeptide"
QLQLQESGPGLVKPSETLSLTCTVSGGSISSSNYFWGWIRQSPGKGLEWIGSIDYSGYTYYNPSLKSRVTISVDTSKNQFSLKLSSVTAADTAVYNCARHKAATADFDYRGQGTLVTVSSGGGGSGGGGSQLQLQESGPGLVKPSETLSLTCTVSGGSISSSNYFWGWIRQSPGKGLEWIGSIDYSGYTYYNPSLKSRVTISVDTSKNQFSLKLSSVTAADTAVYNCARHKAATADFDYRGQGTLVTVSSESKYGPPCPPCPAPEAAGGPSVFLFPPKPKDTLMISRTPEVTCVVVDVSQEDPEVQFNWYVDGVEVHNAKTKPREEQFNSTYRVVSVLTVLHQDWLNGKEYKCKVSNKGLPSSIEKTISKAKGQPREPQVYTLPPSQEEMTKNQVSLSCAVKGFYPSDIAVEWESNGQPENNYKTTPPVLDSDGSFFLVSRLTVDKSRWQEGNVFSCSVMHEALHNHYTQKSLSLSLG

SEQ ID NO: 83 - protein, 355 aa, synthetic construct
  REGION 1..355: note = source = /note="Description of Artificial Sequence: Syntheticpolypeptide"
QVQLVESGGGVVQPGRSLRLSCAASGFSFSRYGMHWVRQAPGKGLEGVAVIWYDGSNRYYADSVKGRFTISRDNSKNTLYLQMNSLRAEDTAVYYCAREPRIGYYYESSGYYSLDYRGQGTLVTVSSESKYGPPCPPCPAPEAAGGPSVFLFPPKPKDTLMISRTPEVTCVVVDVSQEDPEVQFNWYVDGVEVHNAKTKPREEQFNSTYRVVSVLTVLHQDWLNGKEYKCKVSNKGLPSSIEKTISKAKGQPREPQVYTLPPSQEEMTKNQVSLSCAVKGFYPSDIAVEWESNGQPENNYKTTPPVLDSDGSFFLVSRLTVDKSRWQEGNVFSCSVMHEALHNHYTQKSLSLSLG

SEQ ID NO: 84 - protein, 492 aa, synthetic construct
  REGION 1..492: note = source = /note="Description of Artificial Sequence: Syntheticpolypeptide"
QVQLVESGGGVVQPGRSLRLSCAASGFSFSRYGMHWVRQAPGKGLEGVAVIWYDGSNRYYADSVKGRFTISRDNSKNTLYLQMNSLRAEDTAVYYCAREPRIGYYYESSGYYSLDYRGQGTLVTVSSGGGGSGGGGSQVQLVESGGGVVQPGRSLRLSCAASGFSFSRYGMHWVRQAPGKGLEGVAVIWYDGSNRYYADSVKGRFTISRDNSKNTLYLQMNSLRAEDTAVYYCAREPRIGYYYESSGYYSLDYRGQGTLVTVSSESKYGPPCPPCPAPEAAGGPSVFLFPPKPKDTLMISRTPEVTCVVVDVSQEDPEVQFNWYVDGVEVHNAKTKPREEQFNSTYRVVSVLTVLHQDWLNGKEYKCKVSNKGLPSSIEKTISKAKGQPREPQVYTLPPSQEEMTKNQVSLSCAVKGFYPSDIAVEWESNGQPENNYKTTPPVLDSDGSFFLVSRLTVDKSRWQEGNVFSCSVMHEALHNHYTQKSLSLSLG

SEQ ID NO: 85 - protein, 485 aa, synthetic construct
  REGION 1..485: note = source = /note="Description of Artificial Sequence: Syntheticpolypeptide"
QLQLQESGPGLVKPSETLSLTCTVSGGSISSSNYFWGWIRQSPGKGLEWIGSIDYSGYTYYNPSLKSRVTISVDTSKNQFSLKLSSVTAADTAVYNCARHKAATADFDYRGQGTLVTVSSGGGGSGGGGSQVQLVESGGGVVQPGRSLRLSCAASGFSFSRYGMHWVRQAPGKGLEGVAVIWYDGSNRYYADSVKGRFTISRDNSKNTLYLQMNSLRAEDTAVYYCAREPRIGYYYESSGYYSLDYRGQGTLVTVSSESKYGPPCPPCPAPEAAGGPSVFLFPPKPKDTLMISRTPEVTCVVVDVSQEDPEVQFNWYVDGVEVHNAKTKPREEQFNSTYRVVSVLTVLHQDWLNGKEYKCKVSNKGLPSSIEKTISKAKGQPREPQVYTLPPSQEEMTKNQVSLSCAVKGFYPSDIAVEWESNGQPENNYKTTPPVLDSDGSFFLVSRLTVDKSRWQEGNVFSCSVMHEALHNHYTQKSLSLSLG

SEQ ID NO: 86 - protein, 485 aa, synthetic construct
  REGION 1..485: note = source = /note="Description of Artificial Sequence: Syntheticpolypeptide"
QVQLVESGGGVVQPGRSLRLSCAASGFSFSRYGMHWVRQAPGKGLEGVAVIWYDGSNRYYADSVKGRFTISRDNSKNTLYLQMNSLRAEDTAVYYCAREPRIGYYYESSGYYSLDYRGQGTLVTVSSGGGGSGGGGSQLQLQESGPGLVKPSETLSLTCTVSGGSISSSNYFWGWIRQSPGKGLEWIGSIDYSGYTYYNPSLKSRVTISVDTSKNQFSLKLSSVTAADTAVYNCARHKAATADFDYRGQGTLVTVSSESKYGPPCPPCPAPEAAGGPSVFLFPPKPKDTLMISRTPEVTCVVVDVSQEDPEVQFNWYVDGVEVHNAKTKPREEQFNSTYRVVSVLTVLHQDWLNGKEYKCKVSNKGLPSSIEKTISKAKGQPREPQVYTLPPSQEEMTKNQVSLSCAVKGFYPSDIAVEWESNGQPENNYKTTPPVLDSDGSFFLVSRLTVDKSRWQEGNVFSCSVMHEALHNHYTQKSLSLSLG

SEQ ID NO: 87 - protein, 119 aa, synthetic construct
  REGION 1..119: note = source = /note="Description of Artificial Sequence: Syntheticpolypeptide"
EVQVLESGGGLVQPGGSLRLSCAASGFTVSSYGMSWVRQPPGKGMEWVSGIRGSDGSTFYADSVKGRFTISRDNATNTLYLQMNSLRAEDTAVYYCAKQGGNDGPFDYRGQGTLVTVSS

SEQ ID NO: 88 - protein, 119 aa, synthetic construct
  REGION 1..119: note = source = /note="Description of Artificial Sequence: Syntheticpolypeptide"
EVQLLESGGGLVQPGGSLRLSCAASGFTISSYGMSWVRQAPGKGVEWVSGIRGSDGTTYYADSVKGRFTISRDSSRNTLYLQMNSLRAEDTAVYYCAKQGGNDGPFDHRGQGTLVTVSS

SEQ ID NO: 89 - protein, 119 aa, synthetic construct
  REGION 1..119: note = source = /note="Description of Artificial Sequence: Syntheticpolypeptide"
EVQLLESGGGLVQPGGSLRLSCAASGFTVSSYGMSWVRQAPGKGPEWVSGIRGSDGSTYYADSVKGRFTISRDNATNTLYLQMNSLRAEDTAVYYCAKQGGNDGPFDYRGQGTLVTVSS

SEQ ID NO: 90 - protein, 119 aa, synthetic construct
  REGION 1..119: note = source = /note="Description of Artificial Sequence: Syntheticpolypeptide"
EVQLLESGGGLVQPGGSLRLSCAASGFTVSSYGMSWVRQAPGKGPEWVSGIRGSDGSTYYADSVKGRFTISRDNSKNTLYLQMNSLRAEDTAVYYCAKQGENDGPFDHRGQGTLVTVSS

SEQ ID NO: 91 - protein, 119 aa, synthetic construct
  REGION 1..119: note = source = /note="Description of Artificial Sequence: Syntheticpolypeptide"
EVQLLESGGGLVQPGGSLRLSCAASGFTVSSYGMSWVRQPPGKGMEWVSGIRGSDGSTYYADSVKGRFTISRDNAKNTLYLQMNSLRAEDTAVYYCAKQGGNDGPFDYRGQGTLVTVSS

SEQ ID NO: 92 - protein, 119 aa, synthetic construct
  REGION 1..119: note = source = /note="Description of Artificial Sequence: Syntheticpolypeptide"
EVQLLESGGGLVQAGGSLRLSCAASGFTVSSYGMSWVRQAPGKGPEWVSGIRGSDGSTYYADSVKGRFTISRDNSKNTLYLQMNSLRAEDTAVYHCAKQGENDGPFDYRGQGTLVTVSS

SEQ ID NO: 93 - protein, 50 aa, synthetic construct
  SITE 1..50: note = /note="This sequence may encompass 1-10 'Gly Gly Gly Gly Ser'repeating units"
  REGION 1..50: note = source = /note="Description of Artificial Sequence: Syntheticpolypeptide"
  REGION 1..50: note = source = /note="See specification as filed for detailed description ofsubstitutions and preferred embodiments"
GGGGSGGGGSGGGGSGGGGSGGGGSGGGGSGGGGSGGGGSGGGGSGGGGS